European Patent Application EP 4 663 190 A2, published December 17, 2025. Title: Muscarinic receptor agonists. Applicant: Heptares Therapeutics Limited. Application WO PCT/EP2023/071591, filed August 3, 2023. The sequence listing filed with the application follows.

SEQUENCE LISTING (2 sequences)

SEQ ID NO: 1 - protein, 267 aa, synthetic construct
MNSVQSQGTALITGASSGIGAIYAERLAARGFDLLLVARDKARLDSAASQLRDAHGVQVEVWKADLTQKDDVIKLEQRLRSDSSISLLINNAGVAADGPLANADMDQLERLIQLNITAVTRLASAAAASFAKAGRGTIINIASVVALFPERFNATYTASKAYVLSLTQSLNAELEGSGVQIQAVLPGVTRTEIWERSGIDASGIPAEMVMDAGEMVDAALAGLDQGELVTIPSLPDAGEWQSFVAARHVMAPNLSRSAAAQRYKSGH

SEQ ID NO: 2 - DNA, 804 bp, synthetic construct
  source 1..804: mol_type = other DNA
atgaattctgtgcagtctcaaggtacggctctgatcactggcgcctcgtccggtatcggtgcgatttacgccgagcgtctggcggcgcgtggttttgatctgttgctggtggcccgtgacaaggcccgtctggacagcgccgccagccaattgcgcgacgctcacggtgtgcaggtcgaggtgtggaaagcggatctgacccaaaaggacgacgtgatcaaactcgaacagcgcttgcgcagcgattcgagcatcagcctgctgattaacaatgccggcgtggccgccgacggcccgctggccaatgccgacatggatcaactggaacgcctgatccagttgaacatcaccgccgtcacgcgtctggcgtcggccgccgctgccagtttcgccaaggcaggtcgcggcacgatcatcaacatcgcctcggtcgtggcgctgttccccgagcgtttcaatgcgacctacaccgccagcaaggcctatgtgttgagtctgacccaatcgttgaacgcggagctcgaaggctccggcgtgcagatccaggccgtgctgccgggcgtgacccgcactgaaatctgggagcgttcggggatcgacgccagtggcattccggcggaaatggtcatggacgccggggagatggtggatgccgccctggccggtctggatcagggcgaactggtcaccattccatcgctgcccgatgccggcgaatggcagtcgtttgtggcggcgcgccatgtcatggcgccgaacctttcgcgcagcgctgcagcccagcgctacaaatcaggtcattga